European Patent Application EP 4 741 421 A1, published May 13, 2026. Title: 작용기 기능이 제거된 Fab-arm 교환 방지 Fc 변이체들. Applicant: 고려대학교 산학협력단. Application WO. The sequence listing filed with the application follows.

SEQUENCE LISTING (10 sequences)

SEQ ID NO: 1 - protein, 229 aa, synthetic construct
ESKYGPPCPSCPCPEFLGGPSVFLFPPKPKDTLMISRTPEVTCVVVDVSQEDPEVQFNWYVDGVEVHNAKTKPREEQFNSTYRVVSVLTVLHQDWLNGKEYKCKVSNKGLPSSIEKTISKAKGQPREPQVYTLPPSQEEMTKNQVSLTCLVKGFYPSDIAVEWESNGQPENNYKTTPPVLDSDGSFFLYSRLTVDKSRWQEGNVFSCSVMHEALHNHYTQKSLSLSLGK

SEQ ID NO: 2 - DNA, 687 bp, synthetic construct
  source 1..687: mol_type = other DNA
gagagcaagtacggaccaccctgtccttcatgtccttgtcctgagttcctgggcgggccttccgtgttcctgtttcctccaaagccaaaagataccctgatgatctctcggaccccagaggtgacatgcgtggtggtggacgtgagccaggaggatcccgaggtgcagttcaactggtacgtggacggcgtggaggtgcacaatgccaagaccaagcctagggaggagcagtttaacagcacctaccgcgtggtgtccgtgctgacagtgctgcaccaggattggctgaacggcaaggagtataagtgcaaggtgtccaataagggcctgcccagctccatcgagaagaccatctctaaggccaagggccagcctagggagccacaggtgtacacactgccccctagccaggaggagatgaccaagaaccaggtgtccctgacatgtctggtgaagggcttctatccctccgacatcgccgtggagtgggagtctaatggccagcctgagaacaattacaagaccacaccacccgtgctggactccgatggctctttctttctgtattctcggctgacagtggataagagcagatggcaggagggcaacgtgttcagctgtagcgtgatgcacgaagcactgcacaaccattacactcagaaaagcctgtcactgtccctgggcaag

SEQ ID NO: 3 - protein, 229 aa, synthetic construct
ESKYGPPCPSCPACEFLGGPSVFLFPPKPKDTLMISRTPEVTCVVVDVSQEDPEVQFNWYVDGVEVHNAKTKPREEQFNSTYRVVSVLTVLHQDWLNGKEYKCKVSNKGLPSSIEKTISKAKGQPREPQVYTLPPSQEEMTKNQVSLTCLVKGFYPSDIAVEWESNGQPENNYKTTPPVLDSDGSFFLYSRLTVDKSRWQEGNVFSCSVMHEALHNHYTQKSLSLSLGK

SEQ ID NO: 4 - DNA, 687 bp, synthetic construct
  source 1..687: mol_type = other DNA
gagagcaagtacggaccaccctgtccttcatgtcctgcttgtgagttcctgggcgggccttccgtgttcctgtttcctccaaagccaaaagataccctgatgatctctcggaccccagaggtgacatgcgtggtggtggacgtgagccaggaggatcccgaggtgcagttcaactggtacgtggacggcgtggaggtgcacaatgccaagaccaagcctagggaggagcagtttaacagcacctaccgcgtggtgtccgtgctgacagtgctgcaccaggattggctgaacggcaaggagtataagtgcaaggtgtccaataagggcctgcccagctccatcgagaagaccatctctaaggccaagggccagcctagggagccacaggtgtacacactgccccctagccaggaggagatgaccaagaaccaggtgtccctgacatgtctggtgaagggcttctatccctccgacatcgccgtggagtgggagtctaatggccagcctgagaacaattacaagaccacaccacccgtgctggactccgatggctctttctttctgtattctcggctgacagtggataagagcagatggcaggagggcaacgtgttcagctgtagcgtgatgcacgaagcactgcacaaccattacactcagaaaagcctgtcactgtccctgggcaag

SEQ ID NO: 5 - protein, 229 aa, synthetic construct
ESKYGPPCPSCPAPECLGGPSVFLFPPKPKDTLMISRTPEVTCVVVDVSQEDPEVQFNWYVDGVEVHNAKTKPREEQFNSTYRVVSVLTVLHQDWLNGKEYKCKVSNKGLPSSIEKTISKAKGQPREPQVYTLPPSQEEMTKNQVSLTCLVKGFYPSDIAVEWESNGQPENNYKTTPPVLDSDGSFFLYSRLTVDKSRWQEGNVFSCSVMHEALHNHYTQKSLSLSLGK

SEQ ID NO: 6 - DNA, 687 bp, synthetic construct
  source 1..687: mol_type = other DNA
gagagcaagtacggaccaccctgtccttcatgtcctgctcctgagtgtctgggcgggccttccgtgttcctgtttcctccaaagccaaaagataccctgatgatctctcggaccccagaggtgacatgcgtggtggtggacgtgagccaggaggatcccgaggtgcagttcaactggtacgtggacggcgtggaggtgcacaatgccaagaccaagcctagggaggagcagtttaacagcacctaccgcgtggtgtccgtgctgacagtgctgcaccaggattggctgaacggcaaggagtataagtgcaaggtgtccaataagggcctgcccagctccatcgagaagaccatctctaaggccaagggccagcctagggagccacaggtgtacacactgccccctagccaggaggagatgaccaagaaccaggtgtccctgacatgtctggtgaagggcttctatccctccgacatcgccgtggagtgggagtctaatggccagcctgagaacaattacaagaccacaccacccgtgctggactccgatggctctttctttctgtattctcggctgacagtggataagagcagatggcaggagggcaacgtgttcagctgtagcgtgatgcacgaagcactgcacaaccattacactcagaaaagcctgtcactgtccctgggcaag

SEQ ID NO: 7 - protein, 229 aa, synthetic construct
ESKYGPPCPSCPAPEFCGGPSVFLFPPKPKDTLMISRTPEVTCVVVDVSQEDPEVQFNWYVDGVEVHNAKTKPREEQFNSTYRVVSVLTVLHQDWLNGKEYKCKVSNKGLPSSIEKTISKAKGQPREPQVYTLPPSQEEMTKNQVSLTCLVKGFYPSDIAVEWESNGQPENNYKTTPPVLDSDGSFFLYSRLTVDKSRWQEGNVFSCSVMHEALHNHYTQKSLSLSLGK

SEQ ID NO: 8 - DNA, 687 bp, synthetic construct
  source 1..687: mol_type = other DNA
gagagcaagtacggaccaccctgtccttcatgtcctgctcctgagttctgtggcgggccttccgtgttcctgtttcctccaaagccaaaagataccctgatgatctctcggaccccagaggtgacatgcgtggtggtggacgtgagccaggaggatcccgaggtgcagttcaactggtacgtggacggcgtggaggtgcacaatgccaagaccaagcctagggaggagcagtttaacagcacctaccgcgtggtgtccgtgctgacagtgctgcaccaggattggctgaacggcaaggagtataagtgcaaggtgtccaataagggcctgcccagctccatcgagaagaccatctctaaggccaagggccagcctagggagccacaggtgtacacactgccccctagccaggaggagatgaccaagaaccaggtgtccctgacatgtctggtgaagggcttctatccctccgacatcgccgtggagtgggagtctaatggccagcctgagaacaattacaagaccacaccacccgtgctggactccgatggctctttctttctgtattctcggctgacagtggataagagcagatggcaggagggcaacgtgttcagctgtagcgtgatgcacgaagcactgcacaaccattacactcagaaaagcctgtcactgtccctgggcaag

SEQ ID NO: 9 - protein, 229 aa, synthetic construct
ESKYGPPCPSCPAPEFLGGPSVFLFPPKPKDTLMISRTPEVTCVVVDVSQEDPEVQFNWYVDGVEVHNAKTKPREEQFNSTYRVVSVLTVLHQDWLNGKEYKCKVSNKGLPSSIEKTISKAKGQPREPQVYTLPPSQEEMTKNQVSLTCLVKGFYPSDIAVEWESNGQPENNYKTTPPVLDSDGSFFLYSRLTVDKSRWQEGNVFSCSVMHEALHNHYTQKSLSLSLGK

SEQ ID NO: 10 - DNA, 687 bp, synthetic construct
  source 1..687: mol_type = other DNA
gagagcaagtacggaccaccctgtccttcatgtcctgctcctgagttcctgggcgggccttccgtgttcctgtttcctccaaagccaaaagataccctgatgatctctcggaccccagaggtgacatgcgtggtggtggacgtgagccaggaggatcccgaggtgcagttcaactggtacgtggacggcgtggaggtgcacaatgccaagaccaagcctagggaggagcagtttaacagcacctaccgcgtggtgtccgtgctgacagtgctgcaccaggattggctgaacggcaaggagtataagtgcaaggtgtccaataagggcctgcccagctccatcgagaagaccatctctaaggccaagggccagcctagggagccacaggtgtacacactgccccctagccaggaggagatgaccaagaaccaggtgtccctgacatgtctggtgaagggcttctatccctccgacatcgccgtggagtgggagtctaatggccagcctgagaacaattacaagaccacaccacccgtgctggactccgatggctctttctttctgtattctcggctgacagtggataagagcagatggcaggagggcaacgtgttcagctgtagcgtgatgcacgaagcactgcacaaccattacactcagaaaagcctgtcactgtccctgggcaag